European Patent Application EP 4 582 805 A2, published July 9, 2025. Title: METHODS OF GENERATING LIBRARIES OF NUCLEIC ACID SEQUENCES FOR DETECTION VIA FLUORESCENT IN SITU SEQUENCING. Applicant: President and Fellows of Harvard College. Application WO PCT/US2017/049633, filed August 31, 2017. The sequence listing filed with the application follows.

SEQUENCE LISTING (1 sequence)

SEQ ID NO: 1 - DNA, 23 bp, synthetic construct
  misc_feature 1..23: note = Description of Artificial Sequence: Synthetic oligonucleotide
  source 1..23: mol_type = other DNA
acttcagctgccccgggtgaaga